European Patent Application EP 4 620 480 A1, published September 24, 2025. Title: Implantation promoting agent and screening system thereof. Applicant: KANSAI MEDICAL UNIVERSITY. The sequence listing filed with the application follows.

SEQUENCE LISTING (2 sequences)

SEQ ID NO: 1 - protein, 13 aa, synthetic construct
  REGION 1..13: note = Integrin activating peptide 1
KFEEERMRCKWMT

SEQ ID NO: 2 - protein, 13 aa, synthetic construct
  REGION 1..13: note = Integrin activating peptide 2
KFEEERSRCKWMT